European Patent Application EP 4 410 316 A1, published August 7, 2024. Title: Nanoparticles for delivery of nucleic acid cargos. Applicant: 4basebio UK Ltd. Application EP. The sequence listing filed with the application follows.

SEQUENCE LISTING (3 sequences)

SEQ ID NO: 1 - protein, 16 aa, synthetic construct
KKKKKKKKKKKKKKKK

SEQ ID NO: 2 - protein, 30 aa, synthetic construct
KKKKKKKKKKKKKKKKKKKKKKKKKKKKKK

SEQ ID NO: 3 - DNA, 13 bp, synthetic construct
  source 1..13: mol_type = other DNA
aaaaaacataaaa